European Patent Application EP 4 582 449 A1, published July 9, 2025. Title: RECOMBINANT HUMANIZED MONOCLONAL ANTIBODY TARGETING HUMAN GPRC5D AND APPLICATION THEREOF. Applicant: Suzhou Dima Biotechnology Co., Ltd. The sequence listing filed with the application follows.

SEQUENCE LISTING (107 sequences)

SEQ ID NO: 1 - protein, 7 aa, synthetic construct
  source 1..7: note = VH-CDR1
LSSNAMS

SEQ ID NO: 2 - protein, 12 aa, synthetic construct
  source 1..12: note = VH-CDR2
SVGSSGRPYYAN

SEQ ID NO: 3 - protein, 12 aa, synthetic construct
  source 1..12: note = VH-CDR3
FTGGTSGGYFSI

SEQ ID NO: 4 - protein, 13 aa, synthetic construct
  source 1..13: note = VL-CDR1
QASQSVYNNNLLA

SEQ ID NO: 5 - protein, 4 aa, synthetic construct
  source 1..4: note = VL-CDR2
SAST

SEQ ID NO: 6 - protein, 10 aa, synthetic construct
  source 1..10: note = VL-CDR3
QGYYSGAICT

SEQ ID NO: 7 - protein, 120 aa, synthetic construct
  source 1..120: note = G01 VH
EVQLVESGGGLVQPGGSLRLSCTASGFSLSSNAMSWVRQAPGKGLEWIGSVGSSGRPYYANWAKGRFTISRDNSKNTVYLQMNSLRAEDTAVYFCARFTGGTSGGYFSIWGPGTLVTVSS

SEQ ID NO: 8 - DNA, 360 bp, synthetic construct
  source 1..360: mol_type = other DNA; note = G01 VH
gaagtgcagctggtggagtccggcggtggactggtgcaaccgggaggctcactcagattgtcatgcaccgcctctggctttagtctcagtagtaatgcaatgagctgggtgaggcaggcacccggcaagggcctggaatggatcggcagcgttggtagtagtggtagaccatactacgcgaactgggcgaagggcaggtttaccatcagccgcgacaacagcaagaataccgtttacctgcagatgaatagcctgagggccgaagacacggcggtctatttctgtgcacggtttactggtggtactagtgggggttacttttccatctggggccctgggaccctcgtaactgtgagcagc

SEQ ID NO: 9 - protein, 110 aa, synthetic construct
  source 1..110: note = G01 VL
DIQMTQSPSTLSASVGDRVIINCQASQSVYNNNLLAWYQQKPGKAPKLLIYSASTLASGVPSRFSGSGSGAEFTLTISSLQPDDFATYYCQGYYSGAICTFGQGTKLTVL

SEQ ID NO: 10 - DNA, 330 bp, synthetic construct
  source 1..330: mol_type = other DNA; note = G01 VL
gacatccagatgacccagtccccaagtacactgagcgcctccgtgggcgaccgcgtgatcataaactgtcaggccagtcagagtgtttataataacaacctcttagcctggtatcaacagaagcccggtaaggcccccaaactgctcatttactctgcatccactctggcatccggggtgccaagccgcttctccgggagtgggtctggcgccgagttcaccctgaccatatcttccctgcagcccgacgacttcgcaacgtactattgccaaggctactatagtggtgctatttgtactttcgggcagggcacgaagttgaccgtgctg

SEQ ID NO: 11 - protein, 245 aa, synthetic construct
  source 1..245: note = G01 scFv
DIQMTQSPSTLSASVGDRVIINCQASQSVYNNNLLAWYQQKPGKAPKLLIYSASTLASGVPSRFSGSGSGAEFTLTISSLQPDDFATYYCQGYYSGAICTFGQGTKLTVLGGGGSGGGGSGGGGSEVQLVESGGGLVQPGGSLRLSCTASGFSLSSNAMSWVRQAPGKGLEWIGSVGSSGRPYYANWAKGRFTISRDNSKNTVYLQMNSLRAEDTAVYFCARFTGGTSGGYFSIWGPGTLVTVSS

SEQ ID NO: 12 - protein, 12 aa, synthetic construct
  source 1..12: note = VH-CDR2
SIGRSGSTYNAN

SEQ ID NO: 13 - protein, 13 aa, synthetic construct
  source 1..13: note = VH-CDR3
KFTGGVSGGYFSV

SEQ ID NO: 14 - protein, 13 aa, synthetic construct
  source 1..13: note = VL-CDR1
QASQSVYNNNLLS

SEQ ID NO: 15 - protein, 4 aa, synthetic construct
  source 1..4: note = VL-CDR2
AASN

SEQ ID NO: 16 - protein, 10 aa, synthetic construct
  source 1..10: note = VL-CDR3
QGYYGGAICA

SEQ ID NO: 17 - protein, 120 aa, synthetic construct
  source 1..120: note = G02 VH
EVQLVESGGGLVQPGGSLRLSCTASGFSLSSNAMSWVRQAPGKGLEWIGSIGRSGSTYNANWAKGRFTISRDNSKNTVYLQMNSLRAEDTAVYFCAKFTGGVSGGYFSVWGPGTLVTVSS

SEQ ID NO: 18 - DNA, 360 bp, synthetic construct
  source 1..360: mol_type = other DNA; note = G02 VH
gaagtgcagctggtggagtccggcggtggactggtgcaaccgggaggctcactcagattgtcatgcaccgcctctggctttagtctcagtagtaatgcaatgagctgggtgaggcaggcacccggcaagggcctggaatggatcggcagcattggtcgtagtggtagcacatacaacgcgaactgggcgaagggcaggtttaccatcagccgcgacaacagcaagaataccgtttacctgcagatgaatagcctgagggccgaagacacggcggtctatttctgtgcaaaatttactggtggtgttagtgggggttactttagcgtctggggccctgggaccctcgtaactgtgagcagc

SEQ ID NO: 19 - protein, 110 aa, synthetic construct
  source 1..110: note = G02 VL
DIQMTQSPSTLSASVGDRVIINCQASQSVYNNNLLSWYQQKPGKAPKLLIYAASNLASGVPSRFSGSGSGAEFTLTISSLQPDDFATYYCQGYYGGAICAFGQGTKLTVL

SEQ ID NO: 20 - DNA, 330 bp, synthetic construct
  source 1..330: mol_type = other DNA; note = G02 VL
gacatccagatgacccagtccccaagtacactgagcgcctccgtgggcgaccgcgtgatcataaactgtcaggccagtcagagtgtttataataacaacctcttatcttggtatcaacagaagcccggtaaggcccccaaactgctcatttacgctgcatccaatctggcatccggggtgccaagccgcttctccgggagtgggtctggcgccgagttcaccctgaccatatcttccctgcagcccgacgacttcgcaacgtactattgccaaggctactatggtggtgctatttgtgctttcgggcagggcacgaagttgaccgtgctg

SEQ ID NO: 21 - protein, 245 aa, synthetic construct
  source 1..245: note = G02 scFv
DIQMTQSPSTLSASVGDRVIINCQASQSVYNNNLLSWYQQKPGKAPKLLIYAASNLASGVPSRFSGSGSGAEFTLTISSLQPDDFATYYCQGYYGGAICAFGQGTKLTVLGGGGSGGGGSGGGGSEVQLVESGGGLVQPGGSLRLSCTASGFSLSSNAMSWVRQAPGKGLEWIGSIGRSGSTYNANWAKGRFTISRDNSKNTVYLQMNSLRAEDTAVYFCAKFTGGVSGGYFSVWGPGTLVTVSS

SEQ ID NO: 22 - protein, 10 aa, synthetic construct
  source 1..10: note = VH-CDR1
IDFSSSYWIC

SEQ ID NO: 23 - protein, 14 aa, synthetic construct
  source 1..14: note = VH-CDR2
ACIANGDGSTYYAS

SEQ ID NO: 24 - protein, 12 aa, synthetic construct
  source 1..12: note = VH-CDR3
DPYLGYSVQLNL

SEQ ID NO: 25 - protein, 11 aa, synthetic construct
  source 1..11: note = VL-CDR1
QASEDIGNNLA

SEQ ID NO: 26 - protein, 4 aa, synthetic construct
  source 1..4: note = VL-CDR2
KAST

SEQ ID NO: 27 - protein, 14 aa, synthetic construct
  source 1..14: note = VL-CDR3
QCTTYYGSGYGVGA

SEQ ID NO: 28 - protein, 122 aa, synthetic construct
  source 1..122: note = G03 VH
EVQLVESGGGLVQPGGSLRLSCTASGIDFSSSYWICWVRQAPGKGLEWIACIANGDGSTYYASWAKGRFTISRDNSKNTVYLQMNSLRAEDTAVYFCARDPYLGYSVQLNLWGPGTLVTVSS

SEQ ID NO: 29 - DNA, 366 bp, synthetic construct
  source 1..366: mol_type = other DNA; note = G03 VH
gaagtgcagctggtggagtccggcggtggactggtgcaaccgggaggctcactcagattgtcatgcaccgcctctggcatcgacttcagtagcagctactggatatgctgggtgaggcaggcacccggcaagggcctggaatggatcgcatgcattgctaatggtgatggcagcacatactacgcgagctgggcgaagggcaggtttaccatcagccgcgacaacagcaagaataccgtttacctgcagatgaatagcctgagggccgaagacacggcggtctatttctgtgcacgggatccttatcttggttatagtgttcaacttaacttgtggggccctgggaccctcgtaactgtgagcagc

SEQ ID NO: 30 - protein, 112 aa, synthetic construct
  source 1..112: note = G03 VL
DIQMTQSPSTLSASVGDRVIINCQASEDIGNNLAWYQQKPGKAPKLLIYKASTLASGVPSRFSGSGSGAEFTLTISSLQPDDFATYYCQCTTYYGSGYGVGAFGQGTKLTVL

SEQ ID NO: 31 - DNA, 336 bp, synthetic construct
  source 1..336: mol_type = other DNA; note = G03 VL
gacatccagatgacccagtccccaagtacactgagcgcctccgtgggcgaccgcgtgatcataaactgtcaggccagtgaggatattggtaataatttagcctggtatcaacagaagcccggtaaggcccccaaactgctcatttacaaggcatccactctggcatccggggtgccaagccgcttctccgggagtgggtctggcgccgagttcaccctgaccatatcttccctgcagcccgacgacttcgcaacgtactattgccaatgtactacttattatggtagtggttatggggttggggctttcgggcagggcacgaagttgaccgtgctg

SEQ ID NO: 32 - protein, 249 aa, synthetic construct
  source 1..249: note = G03 scFv
DIQMTQSPSTLSASVGDRVIINCQASEDIGNNLAWYQQKPGKAPKLLIYKASTLASGVPSRFSGSGSGAEFTLTISSLQPDDFATYYCQCTTYYGSGYGVGAFGQGTKLTVLGGGGSGGGGSGGGGSEVQLVESGGGLVQPGGSLRLSCTASGIDFSSSYWICWVRQAPGKGLEWIACIANGDGSTYYASWAKGRFTISRDNSKNTVYLQMNSLRAEDTAVYFCARDPYLGYSVQLNLWGPGTLVTVSS

SEQ ID NO: 33 - protein, 7 aa, synthetic construct
  source 1..7: note = VH-CDR1
LSSNAIS

SEQ ID NO: 34 - protein, 12 aa, synthetic construct
  source 1..12: note = VH-CDR2
IITTGGNAYYAG

SEQ ID NO: 35 - protein, 7 aa, synthetic construct
  source 1..7: note = VH-CDR3
GYGIHNF

SEQ ID NO: 36 - protein, 13 aa, synthetic construct
  source 1..13: note = VL-CDR1
KCQASESISNYLS

SEQ ID NO: 37 - protein, 4 aa, synthetic construct
  source 1..4: note = VL-CDR2
RAST

SEQ ID NO: 38 - protein, 15 aa, synthetic construct
  source 1..15: note = VL-CDR3
QGYDGSSSSSNYESA

SEQ ID NO: 39 - protein, 115 aa, synthetic construct
  source 1..115: note = G04 VH
EVQLVESGGGLVQPGGSLRLSCAASGFSLSSNAISWVRQAPGKGLEWIGIITTGGNAYYAGWAKGRFTISRDNSKNTLYLQMNSLRAEDTAVYYCARGYGIHNFWGPGTLVTVSS

SEQ ID NO: 40 - DNA, 345 bp, synthetic construct
  source 1..345: mol_type = other DNA; note = G04 VH
gaagtgcagctggtggagtccggcggtggactggtgcaaccgggaggctcactcagattgtcatgcgccgcctctggctttagtctcagtagcaatgcaatcagctgggtgaggcaggcacccggcaagggcctggaatggatcggcatcattactactggtggtaatgcatactacgcaggctgggcgaagggcaggtttaccatcagccgcgacaacagcaagaataccctgtacctgcagatgaatagcctgagggccgaagacacggcggtctattattgtgcacgggggtatggtattcataacttctggggccctgggaccctcgtaactgtgagcagc

SEQ ID NO: 41 - protein, 113 aa, synthetic construct
  source 1..113: note = G04 VL
DIQMTQSPSSLSASVGDRVTIKCQASESISNYLSWYQQKPGKVPKLLIYRASTLASGVPSRFSGSGSGTDFTLTISSLQPEDVATYYCQGYDGSSSSSNYESAFGQGTKLTVL

SEQ ID NO: 42 - DNA, 339 bp, synthetic construct
  source 1..339: mol_type = other DNA; note = G04 VL
gacatccagatgacccagtccccaagttccctgagcgcctccgtgggcgaccgcgtgaccataaagtgccaggccagtgaaagcattagcaactacttatcctggtatcaacagaagcccggtaaggtgcccaaactgctcatttacagggcatccactctggcatccggggtgccaagccgcttctccgggagtgggtctggcaccgacttcaccctgaccatatcttccctgcagcccgaggacgtggcaacgtactattgccagggctatgatggtagtagtagtagtagtaattatgagagtgctttcgggcagggcacgaagttgaccgtgctg

SEQ ID NO: 43 - protein, 243 aa, synthetic construct
  source 1..243: note = G04 scFv
DIQMTQSPSSLSASVGDRVTIKCQASESISNYLSWYQQKPGKVPKLLIYRASTLASGVPSRFSGSGSGTDFTLTISSLQPEDVATYYCQGYDGSSSSSNYESAFGQGTKLTVLGGGGSGGGGSGGGGSEVQLVESGGGLVQPGGSLRLSCAASGFSLSSNAISWVRQAPGKGLEWIGIITTGGNAYYAGWAKGRFTISRDNSKNTLYLQMNSLRAEDTAVYYCARGYGIHNFWGPGTLVTVSS

SEQ ID NO: 44 - protein, 7 aa, synthetic construct
  source 1..7: note = VH-CDR1
LTDNGIT

SEQ ID NO: 45 - protein, 12 aa, synthetic construct
  source 1..12: note = VH-CDR2
IMTTGGSTYYAG

SEQ ID NO: 46 - protein, 12 aa, synthetic construct
  source 1..12: note = VH-CDR3
TYFCTRGYGIHG

SEQ ID NO: 47 - protein, 11 aa, synthetic construct
  source 1..11: note = VL-CDR1
QASESISKFLS

SEQ ID NO: 48 - protein, 15 aa, synthetic construct
  source 1..15: note = VL-CDR3
QGYDGSSTTTNYESA

SEQ ID NO: 49 - protein, 115 aa, synthetic construct
  source 1..115: note = G05 VH
EVQLVESGGGLVQPGGSLRLSCAASGFSLTDNGITWVRQAPGKGLEWIGIMTTGGSTYYAGWAKGRFTISRDNSKNTLYLQMNSLRAEDTATYFCTRGYGIHGLWGPGTLVTVSS

SEQ ID NO: 50 - DNA, 346 bp, synthetic construct
  source 1..346: mol_type = other DNA; note = G05 VH
gaagtgcagctggtggagtccggcggtggactggtgcaaccgggaggctcactcagattgtcatgcgccgcctctggctttagtctcactgacaatggaataacctgggtgaggcaggcacccggcaagggcctggaatggatcggcattatgactactggtggtagcacatactacgcaggctgggcgaagggcaggtttaccatcagccgcgacaacagcaagaataccctgtacctgcagatgaatagcctgagggccgaagacacggcgacctatttctgtaccagagggtatggcattcatggtctgtggggccctgggaccctcgtaactgtgagcagca

SEQ ID NO: 51 - protein, 113 aa, synthetic construct
  source 1..113: note = G05 VL
DIQMTQSPSSLSASVGDRVTITCQASESISKFLSWYQQKPGKVPKLLIYRASTLASGVPSRFSGSGSGTDFTLTISSLQPEDVATYYCQGYDGSSTTTNYESAFGQGTKLTVL

SEQ ID NO: 52 - DNA, 339 bp, synthetic construct
  source 1..339: mol_type = other DNA; note = G05 VL
gacatccagatgacccagtccccaagttccctgagcgcctccgtgggcgaccgcgtgaccataacctgtcaggccagtgagagtattagtaagttcttatcctggtatcaacagaagcccggtaaggtgcccaaactgctcatttacagggcatccactctggcatccggggtgccaagccgcttctccgggagtgggtctggcaccgacttcaccctgaccatatcttccctgcagcccgaggacgtggcaacgtactattgccaaggttatgatggtagtagtactactactaattatgagagtgctttcgggcagggcacgaagttgaccgtgctg

SEQ ID NO: 53 - protein, 243 aa, synthetic construct
  source 1..243: note = G05 scFv
DIQMTQSPSSLSASVGDRVTITCQASESISKFLSWYQQKPGKVPKLLIYRASTLASGVPSRFSGSGSGTDFTLTISSLQPEDVATYYCQGYDGSSTTTNYESAFGQGTKLTVLGGGGSGGGGSGGGGSEVQLVESGGGLVQPGGSLRLSCAASGFSLTDNGITWVRQAPGKGLEWIGIMTTGGSTYYAGWAKGRFTISRDNSKNTLYLQMNSLRAEDTATYFCTRGYGIHGLWGPGTLVTVSS

SEQ ID NO: 54 - protein, 12 aa, synthetic construct
  source 1..12: note = VH-CDR2
IMTTGGSAYYAG

SEQ ID NO: 55 - protein, 7 aa, synthetic construct
  source 1..7: note = VH-CDR3
TRGYGIH

SEQ ID NO: 56 - protein, 116 aa, synthetic construct
  source 1..116: note = G06 VH
EVQLVESGGGLVQPGGSLRLSCAASGFSLTDNGITWVRQAPGKGLEWIGIMTTGGSAYYAGWAKGRFTISRDNSKNTLYLQMNSLRAEDTAVYYCARTRGYGIHLWGPGTLVTVSS

SEQ ID NO: 57 - DNA, 348 bp, synthetic construct
  source 1..348: mol_type = other DNA; note = G06 VH
gaagtgcagctggtggagtccggcggtggactggtgcaaccgggaggctcactcagattgtcatgcgccgcctctggctttagtctcactgacaatggaataacctgggtgaggcaggcacccggcaagggcctggaatggatcggcattatgactactggtggtagcgcatactacgcaggctgggcgaagggcaggtttaccatcagccgcgacaacagcaagaataccctgtacctgcagatgaatagcctgagggccgaagacacggcggtctattattgtgcacggaccagagggtatggcattcatctgtggggccctgggaccctcgtaactgtgagcagc

SEQ ID NO: 58 - protein, 244 aa, synthetic construct
  source 1..244: note = G06 scFv
DIQMTQSPSSLSASVGDRVTITCQASESISKFLSWYQQKPGKVPKLLIYRASTLASGVPSRFSGSGSGTDFTLTISSLQPEDVATYYCQGYDGSSTTTNYESAFGQGTKLTVLGGGGSGGGGSGGGGSEVQLVESGGGLVQPGGSLRLSCAASGFSLTDNGITWVRQAPGKGLEWIGIMTTGGSAYYAGWAKGRFTISRDNSKNTLYLQMNSLRAEDTAVYYCARTRGYGIHLWGPGTLVTVSS

SEQ ID NO: 59 - protein, 12 aa, synthetic construct
  source 1..12: note = VH-CDR2
IMTTGGTTYYAG

SEQ ID NO: 60 - protein, 6 aa, synthetic construct
  source 1..6: note = VH-CDR3
GYGIHG

SEQ ID NO: 61 - protein, 11 aa, synthetic construct
  source 1..11: note = VL-CDR1
QASESVSKFLS

SEQ ID NO: 62 - protein, 115 aa, synthetic construct
  source 1..115: note = G07 VH
EVQLVESGGGLVQPGGSLRLSCAASGFSLTDNGITWVRQAPGKGLEWIGIMTTGGTTYYAGWAKGRFTISRDNSKNTLYLQMNSLRAEDTAVYYCARGYGIHGLWGPGTLVTVSS

SEQ ID NO: 63 - DNA, 345 bp, synthetic construct
  source 1..345: mol_type = other DNA; note = G07 VH
gaagtgcagctggtggagtccggcggtggactggtgcaaccgggaggctcactcagattgtcatgcgccgcctctggctttagtctcactgacaatggaataacctgggtgaggcaggcacccggcaagggcctggaatggatcggcattatgactactggtggtaccacatactacgcaggctgggcgaagggcaggtttaccatcagccgcgacaacagcaagaataccctgtacctgcagatgaatagcctgagggccgaagacacggcggtctattattgtgcacgggggtatggcattcatggtctgtggggccctgggaccctcgtaactgtgagcagc

SEQ ID NO: 64 - protein, 113 aa, synthetic construct
  source 1..113: note = G07 VL
DIQMTQSPSSLSASVGDRVTITCQASESVSKFLSWYQQKPGKVPKLLIYRASTLASGVPSRFSGSGSGTDFTLTISSLQPEDVATYYCQGYDGSSTTTNYESAFGQGTKLTVL

SEQ ID NO: 65 - DNA, 339 bp, synthetic construct
  source 1..339: mol_type = other DNA; note = G07 VL
gacatccagatgacccagtccccaagttccctgagcgcctccgtgggcgaccgcgtgaccataacctgtcaggccagtgaaagcgttagtaagttcttatcctggtatcaacagaagcccggtaaggtgcccaaactgctcatttacagggcatccactctggcatccggggtgccaagccgcttctccgggagtgggtctggcaccgacttcaccctgaccatatcttccctgcagcccgaggacgtggcaacgtactattgccaaggttatgatggtagtagtactactactaattatgagagtgctttcgggcagggcacgaagttgaccgtgctg

SEQ ID NO: 66 - protein, 243 aa, synthetic construct
  source 1..243: note = G07 scFv
DIQMTQSPSSLSASVGDRVTITCQASESVSKFLSWYQQKPGKVPKLLIYRASTLASGVPSRFSGSGSGTDFTLTISSLQPEDVATYYCQGYDGSSTTTNYESAFGQGTKLTVLGGGGSGGGGSGGGGSEVQLVESGGGLVQPGGSLRLSCAASGFSLTDNGITWVRQAPGKGLEWIGIMTTGGTTYYAGWAKGRFTISRDNSKNTLYLQMNSLRAEDTAVYYCARGYGIHGLWGPGTLVTVSS

SEQ ID NO: 67 - protein, 7 aa, synthetic construct
  source 1..7: note = VH-CDR1
LSTYAVS

SEQ ID NO: 68 - protein, 12 aa, synthetic construct
  source 1..12: note = VH-CDR2
IISRSGNTYYAS

SEQ ID NO: 69 - protein, 16 aa, synthetic construct
  source 1..16: note = VH-CDR3
PRIFNSGDIAYLSRLD

SEQ ID NO: 70 - protein, 12 aa, synthetic construct
  source 1..12: note = VL-CDR1
QASQSVYSNALS

SEQ ID NO: 71 - protein, 4 aa, synthetic construct
  source 1..4: note = VL-CDR2
DAST

SEQ ID NO: 72 - protein, 11 aa, synthetic construct
  source 1..11: note = VL-CDR3
AGGYNSIVDNP

SEQ ID NO: 73 - protein, 125 aa, synthetic construct
  source 1..125: note = G08 VH
EVQLVESGGGLVQPGGSLRLSCAASGFSLSTYAVSWVRQAPGKGLEWIGIISRSGNTYYASWAKGRFTISRDNSKNTLYLQMNSLRAEDTAVYYCARPRIFNSGDIAYLSRLDLWGPGTLVTVSS

SEQ ID NO: 74 - DNA, 375 bp, synthetic construct
  source 1..375: mol_type = other DNA; note = G08 VH
gaagtgcagctggtggagtccggcggtggactggtgcaaccgggaggctcactcagattgtcatgcgccgcctctggctttagtctcagtacctatgcagtgagctgggtgaggcaggcacccggcaagggcctggaatggatcggcatcattagtcgtagtggtaacacatactacgcgagctgggcgaagggcaggtttaccatcagccgcgacaacagcaagaataccctgtacctgcagatgaatagcctgagggccgaagacacggcggtctattattgtgcacggccaaggatatttaatagtggtgatattgcctatctaagtcggttggatctgtggggccctgggaccctcgtaactgtgagcagc

SEQ ID NO: 75 - protein, 110 aa, synthetic construct
  source 1..110: note = G08 VL
DIQMTQSPSSLSASVGDRVTITCQASQSVYSNALSWYQQKPGKVPKLLIYDASTLASGVPSRFSGSGSGTDFTLTISSLQPEDVATYYCAGGYNSIVDNPFGQGTKLTVL

SEQ ID NO: 76 - DNA, 330 bp, synthetic construct
  source 1..330: mol_type = other DNA; note = G08 VL
gacatccagatgacccagtccccaagttccctgagcgcctccgtgggcgaccgcgtgaccataacctgtcaggccagtcagagtgtttatagtaacgccttatcctggtatcaacagaagcccggtaaggtgcccaaactgctcatttacgatgcatccactctggcatccggggtgccaagccgcttctccgggagtgggtctggcaccgacttcaccctgaccatatcttccctgcagcccgaggacgtggcaacgtactattgcgcaggcggttacaatagtattgttgataatcctttcgggcagggcacgaagttgaccgtgctg

SEQ ID NO: 77 - protein, 250 aa, synthetic construct
  source 1..250: note = G08 scFv
DIQMTQSPSSLSASVGDRVTITCQASQSVYSNALSWYQQKPGKVPKLLIYDASTLASGVPSRFSGSGSGTDFTLTISSLQPEDVATYYCAGGYNSIVDNPFGQGTKLTVLGGGGSGGGGSGGGGSEVQLVESGGGLVQPGGSLRLSCAASGFSLSTYAVSWVRQAPGKGLEWIGIISRSGNTYYASWAKGRFTISRDNSKNTLYLQMNSLRAEDTAVYYCARPRIFNSGDIAYLSRLDLWGPGTLVTVSS

SEQ ID NO: 78 - protein, 7 aa, synthetic construct
  source 1..7: note = VH-CDR1
LSNNGIT

SEQ ID NO: 79 - protein, 12 aa, synthetic construct
  source 1..12: note = VH-CDR2
IITTTGSAYYAG

SEQ ID NO: 80 - protein, 11 aa, synthetic construct
  source 1..11: note = VL-CDR1
QASESISNYLS

SEQ ID NO: 81 - protein, 15 aa, synthetic construct
  source 1..15: note = VL-CDR3
QGYDGSASSSNYESA

SEQ ID NO: 82 - protein, 115 aa, synthetic construct
  source 1..115: note = G08 VH
EVQLVESGGGLVQPGGSLRLSCAASGFSLSNNGITWVRQAPGKGLEWIGIITTTGSAYYAGWAKGRFTISRDNSKNTLYLQMNSLRAEDTAVYYCARGYGIHGLWGPGTLVTVSS

SEQ ID NO: 83 - DNA, 345 bp, synthetic construct
  source 1..345: mol_type = other DNA; note = G09 VH
gaagtgcagctggtggagtccggcggtggactggtgcaaccgggaggctcactcagattgtcatgcgccgcctctggctttagtctcagtaacaatggaataacctgggtgaggcaggcacccggcaagggcctggaatggatcggcattattactactactggtagcgcatactacgcaggctgggcgaagggcaggtttaccatcagccgcgacaacagcaagaataccctgtacctgcagatgaatagcctgagggccgaagacacggcggtctattattgtgcacgggggtatggtattcatggtctgtggggccctgggaccctcgtaactgtgagcagc

SEQ ID NO: 84 - protein, 113 aa, synthetic construct
  source 1..113: note = G09 VL
DIQMTQSPSSLSASVGDRVTITCQASESISNYLSWYQQKPGKVPKLLIYRASTLASGVPSRFSGSGSGTDFTLTISSLQPEDVATYYCQGYDGSASSSNYESAFGQGTKLTVL

SEQ ID NO: 85 - DNA, 339 bp, synthetic construct
  source 1..339: mol_type = other DNA; note = G09 VL
gacatccagatgacccagtccccaagttccctgagcgcctccgtgggcgaccgcgtgaccataacctgtcaggccagtgaaagcattagcaactacttatcctggtatcaacagaagcccggtaaggtgcccaaactgctcatttacagggcatccactctggcatccggggtgccaagccgcttctccgggagtgggtctggcaccgacttcaccctgaccatatcttccctgcagcccgaggacgtggcaacgtactattgccaaggttatgatggtagtgctagtagtagtaattatgagagtgctttcgggcagggcacgaagttgaccgtgctg

SEQ ID NO: 86 - protein, 243 aa, synthetic construct
  source 1..243: note = G09 scFv
DIQMTQSPSSLSASVGDRVTITCQASESISNYLSWYQQKPGKVPKLLIYRASTLASGVPSRFSGSGSGTDFTLTISSLQPEDVATYYCQGYDGSASSSNYESAFGQGTKLTVLGGGGSGGGGSGGGGSEVQLVESGGGLVQPGGSLRLSCAASGFSLSNNGITWVRQAPGKGLEWIGIITTTGSAYYAGWAKGRFTISRDNSKNTLYLQMNSLRAEDTAVYYCARGYGIHGLWGPGTLVTVSS

SEQ ID NO: 87 - protein, 8 aa, synthetic construct
  source 1..8: note = VH-CDR1
DINSYNMQ

SEQ ID NO: 88 - protein, 12 aa, synthetic construct
  source 1..12: note = VH-CDR2
IIVTGGSRWYAS

SEQ ID NO: 89 - protein, 4 aa, synthetic construct
  source 1..4: note = VH-CDR3
GSAL

SEQ ID NO: 90 - protein, 15 aa, synthetic construct
  source 1..15: note = VL-CDR1
TITCQASESIYSALA

SEQ ID NO: 91 - protein, 14 aa, synthetic construct
  source 1..14: note = VL-CDR3
QSTYYSSSSSYLNT

SEQ ID NO: 92 - protein, 112 aa, synthetic construct
  source 1..112: note = G10 VH
EVQLVESGGGLVQPGGSLRLSCAASGFDINSYNMQWVRQAPGKGLEWIGIIVTGGSRWYASWAKGRFTISRDNSKNTLYLQMNSLRAEDTAVYYCARGSALWGPGTLVTVSS

SEQ ID NO: 93 - DNA, 336 bp, synthetic construct
  source 1..336: mol_type = other DNA; note = G10 VH
gaagtgcagctggtggagtccggcggtggactggtgcaaccgggaggctcactcagattgtcatgcgccgcctctggctttgacatcaatagctacaacatgcaatgggtgaggcaggcacccggcaagggcctggaatggatcggcatcattgttactggtggtagtagatggtacgcgagctgggcgaagggcaggtttaccatcagccgcgacaacagcaagaataccctgtacctgcagatgaatagcctgagggccgaagacacggcggtctattattgtgcacggggatctgccttgtggggccctgggaccctcgtaactgtgagcagc

SEQ ID NO: 94 - protein, 112 aa, synthetic construct
  source 1..112: note = G10 VL
DIQMTQSPSSLSASVGDRVTITCQASESIYSALAWYQQKPGKVPKLLIYKASTLASGVPSRFSGSGSGTDFTLTISSLQPEDVATYYCQSTYYSSSSSYLNTFGQGTKLTVL

SEQ ID NO: 95 - DNA, 336 bp, synthetic construct
  source 1..336: mol_type = other DNA; note = G10 VL
gacatccagatgacccagtccccaagttccctgagcgcctccgtgggcgaccgcgtgaccataacctgtcaggccagtgagagcatttacagtgctttggcctggtatcaacagaagcccggtaaggtgcccaaactgctcatttacaaggcatccactctggcatccggggtgccaagccgcttctccgggagtgggtctggcaccgacttcaccctgaccatatcttccctgcagcccgaggacgtggcaacgtactattgccaaagtacttattatagtagtagtagtagttatcttaatactttcgggcagggcacgaagttgaccgtgctg

SEQ ID NO: 96 - protein, 239 aa, synthetic construct
  source 1..239: note = G10 scFv
DIQMTQSPSSLSASVGDRVTITCQASESIYSALAWYQQKPGKVPKLLIYKASTLASGVPSRFSGSGSGTDFTLTISSLQPEDVATYYCQSTYYSSSSSYLNTFGQGTKLTVLGGGGSGGGGSGGGGSEVQLVESGGGLVQPGGSLRLSCAASGFDINSYNMQWVRQAPGKGLEWIGIIVTGGSRWYASWAKGRFTISRDNSKNTLYLQMNSLRAEDTAVYYCARGSALWGPGTLVTVSS

SEQ ID NO: 97 - protein, 125 aa, synthetic construct
  source 1..125: note = CD3 VH
EVQLLESGGGLVQPGGSLRLSCAASGFTFSTYAMNWVRQAPGKGLEWVSRIRSKYNNYATYYADSVKGRFTISRDDSKNTLYLQMNSLRAEDTAVYYCVRHGNFGNSYVSWFAYWGQGTLVTVSS

SEQ ID NO: 98 - protein, 109 aa, synthetic construct
  source 1..109: note = CD3 VL
QAVVTQEPSLTVSPGGTVTLTCGSSTGAVTTSNYANWVQEKPGQAFRGLIGGTNKRAPGTPARFSGSLLGGKAALTLSGAQPEDEAEYYCALWYSNLWVFGGGTKLTVL

SEQ ID NO: 99 - DNA, 375 bp, synthetic construct
  source 1..375: mol_type = other DNA; note = CD3 VH
gaggtgcaactgctggaaagcggcggaggactcgtgcagcccggcggcagcctgagactgtcttgtgccgccagcggatttacattcagcacctacgccatgaactgggtcagacaggcccctggcaagggcctggaatgggtgtccagaatcagaagcaagtacaacaactacgctacatactatgctgatagcgtgaagggcagattcaccatcagccgggacgacagcaaaaacaccctgtacctgcagatgaattctctgcgggccgaggacaccgccgtgtactactgcgtgcggcacggcaacttcggcaatagctacgtgtcctggttcgcctactggggccagggcaccctggttacagtgtctagc

SEQ ID NO: 100 - DNA, 327 bp, synthetic construct
  source 1..327: mol_type = other DNA; note = CD3 VL
caagccgtggtgacacaggaacccagcctgaccgtgtccccaggcggaacagtgaccctcacctgtggctcttctacaggcgctgtgaccaccagcaactacgccaactgggtgcaggaaaagcccggccaggccttcagaggcctgatcggcggcacaaacaagcgggcccctggcacccctgccagattcagcggcagcctgctgggcggaaaagccgctctgaccctgagcggcgcccagcctgaggacgaggccgagtactactgcgccctgtggtatagcaatctgtgggtctttggcggaggaaccaagctgacagtgctg

SEQ ID NO: 101 - protein, 455 aa, synthetic construct
  source 1..455: note = CD3 VH-Knob
EVQLLESGGGLVQPGGSLRLSCAASGFTFSTYAMNWVRQAPGKGLEWVSRIRSKYNNYATYYADSVKGRFTISRDDSKNTLYLQMNSLRAEDTAVYYCVRHGNFGNSYVSWFAYWGQGTLVTVSSASTKGPSVFPLAPSSKSTSGGTAALGCLVKDYFPEPVTVSWNSGALTSGVHTFPAVLQSSGLYSLSSVVTVPSSSLGTQTYICNVNHKPSNTKVDKKVEPKSCDKTHTCPPCPAPELLGGPSVFLFPPKPKDTLMISRTPEVTCVVVDVSHEDPEVKFNWYVDGVEVHNAKTKPREEQYNSTYRVVSVLTVLHQDWLNGKEYKCKVSNKALPAPIEKTISKAKGQPREPQVYTLPPCREEMTKNQVSLWCLVKGFYPSDIAVEWESNGQPENNYKTTPPVLDSDGSFFLYSKLTVDKSRWQQGNVFSCSVMHEALHNHYTQKSLSLSPGK

SEQ ID NO: 102 - protein, 470 aa, synthetic construct
  source 1..470: note = G05-Hole
DIQMTQSPSSLSASVGDRVTITCQASESISKFLSWYQQKPGKVPKLLIYRASTLASGVPSRFSGSGSGTDFTLTISSLQPEDVATYYCQGYDGSSTTTNYESAFGQGTKLTVLGGGGSGGGGSGGGGSEVQLVESGGGLVQPGGSLRLSCAASGFSLTDNGITWVRQAPGKGLEWIGIMTTGGSTYYAGWAKGRFTISRDNSKNTLYLQMNSLRAEDTATYFCTRGYGIHGLWGPGTLVTVSSDKTHTCPPCPAPELLGGPSVFLFPPKPKDTLMISRTPEVTCVVVDVSHEDPEVKFNWYVDGVEVHNAKTKPREEQYNSTYRVVSVLTVLHQDWLNGKEYKCKVSNKALPAPIEKTISKAKGQPREPQVCTLPPSREEMTKNQVSLSCAVKGFYPSDIAVEWESNGQPENNYKTTPPVLDSDGSFFLVSKLTVDKSRWQQGNVFSCSVMHEALHNHYTQKSLSLSPGK

SEQ ID NO: 103 - protein, 470 aa, synthetic construct
  source 1..470: note = G07-Hole
DIQMTQSPSSLSASVGDRVTITCQASESVSKFLSWYQQKPGKVPKLLIYRASTLASGVPSRFSGSGSGTDFTLTISSLQPEDVATYYCQGYDGSSTTTNYESAFGQGTKLTVLGGGGSGGGGSGGGGSEVQLVESGGGLVQPGGSLRLSCAASGFSLTDNGITWVRQAPGKGLEWIGIMTTGGTTYYAGWAKGRFTISRDNSKNTLYLQMNSLRAEDTAVYYCARGYGIHGLWGPGTLVTVSSDKTHTCPPCPAPELLGGPSVFLFPPKPKDTLMISRTPEVTCVVVDVSHEDPEVKFNWYVDGVEVHNAKTKPREEQYNSTYRVVSVLTVLHQDWLNGKEYKCKVSNKALPAPIEKTISKAKGQPREPQVCTLPPSREEMTKNQVSLSCAVKGFYPSDIAVEWESNGQPENNYKTTPPVLDSDGSFFLVSKLTVDKSRWQQGNVFSCSVMHEALHNHYTQKSLSLSPGK

SEQ ID NO: 104 - protein, 470 aa, synthetic construct
  source 1..470: note = G09-Hole
DIQMTQSPSSLSASVGDRVTITCQASESISNYLSWYQQKPGKVPKLLIYRASTLASGVPSRFSGSGSGTDFTLTISSLQPEDVATYYCQGYDGSASSSNYESAFGQGTKLTVLGGGGSGGGGSGGGGSEVQLVESGGGLVQPGGSLRLSCAASGFSLSNNGITWVRQAPGKGLEWIGIITTTGSAYYAGWAKGRFTISRDNSKNTLYLQMNSLRAEDTAVYYCARGYGIHGLWGPGTLVTVSSDKTHTCPPCPAPELLGGPSVFLFPPKPKDTLMISRTPEVTCVVVDVSHEDPEVKFNWYVDGVEVHNAKTKPREEQYNSTYRVVSVLTVLHQDWLNGKEYKCKVSNKALPAPIEKTISKAKGQPREPQVCTLPPSREEMTKNQVSLSCAVKGFYPSDIAVEWESNGQPENNYKTTPPVLDSDGSFFLVSKLTVDKSRWQQGNVFSCSVMHEALHNHYTQKSLSLSPGK

SEQ ID NO: 105 - protein, 486 aa, synthetic construct
  source 1..486: note = G00-Hole
QSALTQPASVSGSPGQSITISCTGTSSDVGGYNYVSWYQQHPGKAPKLMIYDVSKRPSGVSNRFSGSKSGNTASLTISGLQAEDEADYYCSSYTRSSTEVFGGGTKLTVLGSRGGGGSGGGGSGGGGSLEMAEVQLVQSGAEVKKPGASVKVSCKASGYTFTSYYMHWVRQAPGQGLEWMGIINPSGGSTSYAQKFQGRVTMTRDTSTSTVYMELSSLRSEDTAVYYCARGGSKKWSGEKWRRENFDYWGQGTLVTVSSDKTHTCPPCPAPELLGGPSVFLFPPKPKDTLMISRTPEVTCVVVDVSHEDPEVKFNWYVDGVEVHNAKTKPREEQYNSTYRVVSVLTVLHQDWLNGKEYKCKVSNKALPAPIEKTISKAKGQPREPQVCTLPPSREEMTKNQVSLSCAVKGFYPSDIAVEWESNGQPENNYKTTPPVLDSDGSFFLVSKLTVDKSRWQQGNVFSCSVMHEALHNHYTQKSLSLSPGK

SEQ ID NO: 106 - protein, 220 aa, synthetic construct
  source 1..220: note = Knob
PCPAPELLGGPSVFLFPPKPKDTLMISRTPEVTCVVVDVSHEDPEVKFNWYVDGVEVHNAKTKPREEQYNSTYRVVSVLTVLHQDWLNGKEYKCKVSNKALPAPIEKTISKAKGQPREPQVYTLPPCREEMTKNQVSLWCLVKGFYPSDIAVEWESNGQPENNYKTTPPVLDSDGSFFLYSKLTVDKSRWQQGNVFSCSVMHEALHNHYTQKSLSLSPGK

SEQ ID NO: 107 - protein, 220 aa, synthetic construct
  source 1..220: note = Hole
PCPAPELLGGPSVFLFPPKPKDTLMISRTPEVTCVVVDVSHEDPEVKFNWYVDGVEVHNAKTKPREEQYNSTYRVVSVLTVLHQDWLNGKEYKCKVSNKALPAPIEKTISKAKGQPREPQVCTLPPSREEMTKNQVSLSCAVKGFYPSDIAVEWESNGQPENNYKTTPPVLDSDGSFFLVSKLTVDKSRWQQGNVFSCSVMHEALHNHYTQKSLSLSPGK